European Patent Application EP 4 115 951 A1, published January 11, 2023. Title: CO-STIMULATORY DOMAINS FOR USE IN GENETICALLY-MODIFIED CELLS. Applicant: Precision Biosciences, Inc. The sequence listing filed with the application follows.

SEQUENCE LISTING (42 sequences)

SEQ ID NO: 1 - DNA, 126 bp, Artificial Sequence
  Synthesized
aaacatagccgcaaaaaatttgtgcatctgctgaaacgcccgtttattaaaaccaccggcgcggcgcagatggaagatgcgagcagctgccgctgcccgcaggaagaagaaggcgaatgcgatctg

SEQ ID NO: 2 - DNA, 126 bp, Artificial Sequence
  Synthesized
aaatggggccgcaaaaaactgctgtatctgtttaaacgcccgtttgcgcagccgattcgcaccgcgcaggaagaagatgcgagcagctgccgctttccggaagaagaagaaggcaactgcgaactg

SEQ ID NO: 3 - DNA, 126 bp, Artificial Sequence
  Synthesized
aaacatagccgcaaaaaaattatttttctgtataaaaacccgtttatgaaaccgaccaacagcgcgcaggaagaagatgcgagcagctgccgctttccgcaggaagaagaaggcgattgcgatctg

SEQ ID NO: 4 - DNA, 126 bp, Artificial Sequence
  Synthesized
aaagcgagccgcaaaaaagcggcggcggcggcgaaaagcccgtttgcgagcccggcgagcagcgcgcaggaagaagatgcgagcagctgccgcgcgccgagcgaagaagaaggcagctgcgaactg

SEQ ID NO: 5 - protein, 42 aa, Artificial Sequence
  Synthesized
KHSRKKFVHLLKRPFIKTTGAAQMEDASSCRCPQEEEGECDL

SEQ ID NO: 6 - protein, 42 aa, Artificial Sequence
  Synthesized
KWGRKKLLYLFKRPFAQPIRTAQEEDASSCRFPEEEEGNCEL

SEQ ID NO: 7 - protein, 42 aa, Artificial Sequence
  Synthesized
KHSRKKIIFLYKNPFMKPTNSAQEEDASSCRFPQEEEGDCDL

SEQ ID NO: 8 - protein, 42 aa, Artificial Sequence
  Synthesized
KASRKKAAAAAKSPFASPASSAQEEDASSCRAPSEEEGSCEL

SEQ ID NO: 9 - protein, 4 aa, Artificial Sequence
  Synthesized
QMED

SEQ ID NO: 10 - protein, 4 aa, Artificial Sequence
  Synthesized
QEED

SEQ ID NO: 11 - protein, 4 aa, Artificial Sequence
  Synthesized
EEEG

SEQ ID NO: 12 - protein, 8 aa, Artificial Sequence
  Synthesized
ASSCRCPQ

SEQ ID NO: 13 - protein, 8 aa, Artificial Sequence
  Synthesized
ASSCRFPE

SEQ ID NO: 14 - protein, 8 aa, Artificial Sequence
  Synthesized
ASSCRFPQ

SEQ ID NO: 15 - protein, 8 aa, Artificial Sequence
  Synthesized
ASSCRAPS

SEQ ID NO: 16 - protein, 21 aa, Artificial Sequence
  Synthesized
MALPVTALLLPLALLLHAARP

SEQ ID NO: 17 - protein, 242 aa, Artificial Sequence
  Synthesized
DIQMTQTTSSLSASLGDRVTISCRASQDISKYLNWYQQKPDGTVKLLIYHTSRLHSGVPSRFSGSGSGTDYSLTISNLEQEDIATYFCQQGNTLPYTFGGGTKLEITGGGGSGGGGSGGGGSEVKLQESGPGLVAPSQSLSVTCTVSGVSLPDYGVSWIRQPPRKGLEWLGVIWGSETTYYNSALKSRLTIIKDNSKSQVFLKMNSLQTDDTAIYYCAKHYYYGGSYAMDYWGQGTSVTVSS

SEQ ID NO: 18 - protein, 69 aa, Artificial Sequence
  Synthesized
TTTPAPRPPTPAPTIASQPLSLRPEACRPAAGGAVHTRGLDFACDIYIWAPLAGTCGVLLLSLVITLYC

SEQ ID NO: 19 - protein, 112 aa, Artificial Sequence
  Synthesized
RVKFSRSADAPAYQQGQNQLYNELNLGRREEYDVLDKRRGRDPEMGGKPRRKNPQEGLYNELQKDKMAEAYSEIGMKGERRRGKGHDGLYQGLSTATKDTYDALHMQALPPR

SEQ ID NO: 20 - protein, 41 aa, Artificial Sequence
  Synthesized
RSKRSRLLHSDYMNMTPRRPGPTRKHYQPYAPPRDFAAYRS

SEQ ID NO: 21 - protein, 42 aa, Artificial Sequence
  Synthesized
KRGRKKLLYIFKQPFMRPVQTTQEEDGCSCRFPEEEEGGCEL

SEQ ID NO: 22 - protein, 444 aa, Artificial Sequence
  Synthesized
MALPVTALLLPLALLLHAARPDIQMTQTTSSLSASLGDRVTISCRASQDISKYLNWYQQKPDGTVKLLIYHTSRLHSGVPSRFSGSGSGTDYSLTISNLEQEDIATYFCQQGNTLPYTFGGGTKLEITGGGGSGGGGSGGGGSEVKLQESGPGLVAPSQSLSVTCTVSGVSLPDYGVSWIRQPPRKGLEWLGVIWGSETTYYNSALKSRLTIIKDNSKSQVFLKMNSLQTDDTAIYYCAKHYYYGGSYAMDYWGQGTSVTVSSTTTPAPRPPTPAPTIASQPLSLRPEACRPAAGGAVHTRGLDFACDIYIWAPLAGTCGVLLLSLVITLYCRVKFSRSADAPAYQQGQNQLYNELNLGRREEYDVLDKRRGRDPEMGGKPRRKNPQEGLYNELQKDKMAEAYSEIGMKGERRRGKGHDGLYQGLSTATKDTYDALHMQALPPR

SEQ ID NO: 23 - protein, 485 aa, Artificial Sequence
  Synthesized
MALPVTALLLPLALLLHAARPDIQMTQTTSSLSASLGDRVTISCRASQDISKYLNWYQQKPDGTVKLLIYHTSRLHSGVPSRFSGSGSGTDYSLTISNLEQEDIATYFCQQGNTLPYTFGGGTKLEITGGGGSGGGGSGGGGSEVKLQESGPGLVAPSQSLSVTCTVSGVSLPDYGVSWIRQPPRKGLEWLGVIWGSETTYYNSALKSRLTIIKDNSKSQVFLKMNSLQTDDTAIYYCAKHYYYGGSYAMDYWGQGTSVTVSSTTTPAPRPPTPAPTIASQPLSLRPEACRPAAGGAVHTRGLDFACDIYIWAPLAGTCGVLLLSLVITLYCRSKRSRLLHSDYMNMTPRRPGPTRKHYQPYAPPRDFAAYRSRVKFSRSADAPAYQQGQNQLYNELNLGRREEYDVLDKRRGRDPEMGGKPRRKNPQEGLYNELQKDKMAEAYSEIGMKGERRRGKGHDGLYQGLSTATKDTYDALHMQALPPR

SEQ ID NO: 24 - protein, 486 aa, Artificial Sequence
  Synthesized
MALPVTALLLPLALLLHAARPDIQMTQTTSSLSASLGDRVTISCRASQDISKYLNWYQQKPDGTVKLLIYHTSRLHSGVPSRFSGSGSGTDYSLTISNLEQEDIATYFCQQGNTLPYTFGGGTKLEITGGGGSGGGGSGGGGSEVKLQESGPGLVAPSQSLSVTCTVSGVSLPDYGVSWIRQPPRKGLEWLGVIWGSETTYYNSALKSRLTIIKDNSKSQVFLKMNSLQTDDTAIYYCAKHYYYGGSYAMDYWGQGTSVTVSSTTTPAPRPPTPAPTIASQPLSLRPEACRPAAGGAVHTRGLDFACDIYIWAPLAGTCGVLLLSLVITLYCKRGRKKLLYIFKQPFMRPVQTTQEEDGCSCRFPEEEEGGCELRVKFSRSADAPAYQQGQNQLYNELNLGRREEYDVLDKRRGRDPEMGGKPRRKNPQEGLYNELQKDKMAEAYSEIGMKGERRRGKGHDGLYQGLSTATKDTYDALHMQALPPR

SEQ ID NO: 25 - protein, 486 aa, Artificial Sequence
  Synthesized
MALPVTALLLPLALLLHAARPDIQMTQTTSSLSASLGDRVTISCRASQDISKYLNWYQQKPDGTVKLLIYHTSRLHSGVPSRFSGSGSGTDYSLTISNLEQEDIATYFCQQGNTLPYTFGGGTKLEITGGGGSGGGGSGGGGSEVKLQESGPGLVAPSQSLSVTCTVSGVSLPDYGVSWIRQPPRKGLEWLGVIWGSETTYYNSALKSRLTIIKDNSKSQVFLKMNSLQTDDTAIYYCAKHYYYGGSYAMDYWGQGTSVTVSSTTTPAPRPPTPAPTIASQPLSLRPEACRPAAGGAVHTRGLDFACDIYIWAPLAGTCGVLLLSLVITLYCKHSRKKFVHLLKRPFIKTTGAAQMEDASSCRCPQEEEGECDLRVKFSRSADAPAYQQGQNQLYNELNLGRREEYDVLDKRRGRDPEMGGKPRRKNPQEGLYNELQKDKMAEAYSEIGMKGERRRGKGHDGLYQGLSTATKDTYDALHMQALPPR

SEQ ID NO: 26 - protein, 486 aa, Artificial Sequence
  Synthesized
MALPVTALLLPLALLLHAARPDIQMTQTTSSLSASLGDRVTISCRASQDISKYLNWYQQKPDGTVKLLIYHTSRLHSGVPSRFSGSGSGTDYSLTISNLEQEDIATYFCQQGNTLPYTFGGGTKLEITGGGGSGGGGSGGGGSEVKLQESGPGLVAPSQSLSVTCTVSGVSLPDYGVSWIRQPPRKGLEWLGVIWGSETTYYNSALKSRLTIIKDNSKSQVFLKMNSLQTDDTAIYYCAKHYYYGGSYAMDYWGQGTSVTVSSTTTPAPRPPTPAPTIASQPLSLRPEACRPAAGGAVHTRGLDFACDIYIWAPLAGTCGVLLLSLVITLYCKWGRKKLLYLFKRPFAQPIRTAQEEDASSCRFPEEEEGNCELRVKFSRSADAPAYQQGQNQLYNELNLGRREEYDVLDKRRGRDPEMGGKPRRKNPQEGLYNELQKDKMAEAYSEIGMKGERRRGKGHDGLYQGLSTATKDTYDALHMQALPPR

SEQ ID NO: 27 - protein, 486 aa, Artificial Sequence
  Synthesized
MALPVTALLLPLALLLHAARPDIQMTQTTSSLSASLGDRVTISCRASQDISKYLNWYQQKPDGTVKLLIYHTSRLHSGVPSRFSGSGSGTDYSLTISNLEQEDIATYFCQQGNTLPYTFGGGTKLEITGGGGSGGGGSGGGGSEVKLQESGPGLVAPSQSLSVTCTVSGVSLPDYGVSWIRQPPRKGLEWLGVIWGSETTYYNSALKSRLTIIKDNSKSQVFLKMNSLQTDDTAIYYCAKHYYYGGSYAMDYWGQGTSVTVSSTTTPAPRPPTPAPTIASQPLSLRPEACRPAAGGAVHTRGLDFACDIYIWAPLAGTCGVLLLSLVITLYCKHSRKKIIFLYKNPFMKPTNSAQEEDASSCRFPQEEEGDCDLRVKFSRSADAPAYQQGQNQLYNELNLGRREEYDVLDKRRGRDPEMGGKPRRKNPQEGLYNELQKDKMAEAYSEIGMKGERRRGKGHDGLYQGLSTATKDTYDALHMQALPPR

SEQ ID NO: 28 - protein, 486 aa, Artificial Sequence
  Synthesized
MALPVTALLLPLALLLHAARPDIQMTQTTSSLSASLGDRVTISCRASQDISKYLNWYQQKPDGTVKLLIYHTSRLHSGVPSRFSGSGSGTDYSLTISNLEQEDIATYFCQQGNTLPYTFGGGTKLEITGGGGSGGGGSGGGGSEVKLQESGPGLVAPSQSLSVTCTVSGVSLPDYGVSWIRQPPRKGLEWLGVIWGSETTYYNSALKSRLTIIKDNSKSQVFLKMNSLQTDDTAIYYCAKHYYYGGSYAMDYWGQGTSVTVSSTTTPAPRPPTPAPTIASQPLSLRPEACRPAAGGAVHTRGLDFACDIYIWAPLAGTCGVLLLSLVITLYCKASRKKAAAAAKSPFASPASSAQEEDASSCRAPSEEEGSCELRVKFSRSADAPAYQQGQNQLYNELNLGRREEYDVLDKRRGRDPEMGGKPRRKNPQEGLYNELQKDKMAEAYSEIGMKGERRRGKGHDGLYQGLSTATKDTYDALHMQALPPR

SEQ ID NO: 29 - DNA, 7464 bp, Artificial Sequence
  Synthesized
cagcagctggcgtaatagcgaagaggcccgcaccgatcgcccttcccaacagttgcgcagcctgaatggcgaatggaattccagacgattgagcgtcaaaatgtaggtatttccatgagcgtttttcctgttgcaatggctggcggtaatattgttctggatattaccagcaaggccgatagtttgagttcttctactcaggcaagtgatgttattactaatcaaagaagtattgcgacaacggttaatttgcgtgatggacagactcttttactcggtggcctcactgattataaaaacacttctcaggattctggcgtaccgttcctgtctaaaatccctttaatcggcctcctgtttagctcccgctctgattctaacgaggaaagcacgttatacgtgctcgtcaaagcaaccatagtacgcgccctgtagcggcgcattaagcgcggcgggtgtggtggttacgcgcagcgtgaccgctacacttgccagcgccctagcgcccgctcctttcgctttcttcccttcctttctcgccacgttcgccggctttccccgtcaagctctaaatcgggggctccctttagggttccgatttagtgctttacggcacctcgaccccaaaaaacttgattagggtgatggttcacgtagtgggccatcgccctgatagacggtttttcgccctttgacgttggagtccacgttctttaatagtggactcttgttccaaactggaacaacactcaaccctatctcggtctattcttttgatttataagggattttgccgatttcggcctattggttaaaaaatgagctgatttaacaaaaatttaacgcgaattttaacaaaatattaacgtttacaatttaaatatttgcttatacaatcttcctgtttttggggcttttctgattatcaaccggggtacatatgattgacatgctagttttacggcgcgccgggttggccactccctctctgcgcgctcgctcgctcactgaggccgggcgaccaaaggtcgcccgacgcccgggctttgcccgggcggcctcagtgagcgagcgagcgcgcagagagggagtggccaactccatcactaggggttcctacgcgtagatctcatattctggcagggtcagtggctccaactaacatttgtttggtactttacagtttattaaatagatgtttatatggagaagctctcatttctttctcagaagagcctggctaggaaggtggatgaggcaccatattcattttgcaggtgaaattcctgagatgtaaggagctgctgtgacttgctcaaggccttatatcgagtaaacggtagcgctggggcttagacgcaggtgttctgatttatagttcaaaacctctatcaatgagagagcaatctcctggtaatgtgatagatttcccaacttaatgccaacataccataaacctcccattctgctaatgcccagcctaagttggggagaccactccagattccaagatgtacagtttgctttgctgggcctttttcccatgcctgcctttactctgccagagttatattgctggggttttgaagaagatcctattaaataaaagaataagcagtattattaagtagccctgcatttcaggtttccttgagtggcaggccaggcctggccgtgaacgttcactgaaatcatggcctcttggccaagattgatagcttgtgcctgtccctgagtcccagtccatcacgagcagctggtttctaagatgctatttcccgtataaagcatgagaccgtgacttgccagccccacagagccccgcccttgtccatcactggcatctggactccagcctgggttggggcaaagagggaaatgagatcatgtcctaaccctgatcctcttgtcccacagatatccagaaccctgaccctgccgtgtaccagctgagagactctaaatccagtgacaagtctgtctgcctattcaccgattttgattctcaaacaaatgtgtcacaaagtaaggattctgatgtgtatatcacagacaaaactgtgctagacatgaggtctatggacttcaagagcaacagtgctgtggcctggagcaactagtgggcggagttagggcggagccaatcagcgtgcgccgttccgaaagttgccttttatggctgggcggagaatgggcggtgaacgccgatgattatataaggacgcgccgggtgtggcacagctagttccgtcgcagccgggatttgggtcgcggttcttgtttgttccggaaagccaccatggcgctcccagtgacagccttacttttacctctggcgttattattgcacgcggctcgtcctgacatacagatgactcagactacctcttccctatctgcttctttaggcgaccgagtaacaatatcttgccgggccagccaggacatctcaaaatacttaaactggtatcagcagaagccggacggaacagttaagttgctcatttaccacacgtcgagattacactcaggcgttcctagccgattttcgggttccggttccggtacggactacagcctgacaatcagtaaccttgagcaggaggacatcgccacctacttctgtcagcagggcaacacgctcccgtacacattcggtgggggaactaagctggagattaccggaggcggtggcagcggtggcggcggcagcgggggtggcggctcggaggtcaagttacaggagagcggaccgggcttggtcgcacctagccagagcctctcagtcacgtgcactgtgtctggagtcagtctcccagactacggggtatcatggatacgacagccgcctagaaagggcttagagtggctgggggttatctggggaagtgaaaccacatactacaactcagctctcaagagccgcctcaccatcattaaggacaacagtaagtcgcaggttttcttaaagatgaactctctccagactgacgacaccgctatttactactgcgcgaagcactactactacggcgggagttacgcaatggactactggggtcagggcacttctgtgaccgtatccagcactactaccccagccccacgtccccccacgccagctccaacgatagcaagtcagcccttatctcttcgccctgaggcttgcaggcccgcggcgggcggcgccgttcacacgcgaggactagacttcgcctgcgacatctacatctgggcaccactagccgggacttgcggagtgttgttgttgagcttggtaataacgctctactgcaagcgtgggagaaagaagctcttgtacattttcaagcagccattcatgcgtcccgttcagacgactcaggaggaggacggctgctcgtgccgattcccggaggaggaggagggcggttgcgaactcagagtgaagttctctcgctccgcggacgcacccgcttaccagcagggtcagaaccagctatacaacgagttaaacctggggcgccgggaggagtacgacgtgttagacaagcgtagaggtagggacccggagatgggaggcaagcctcggagaaagaacccccaggagggcctgtacaacgaactccagaaggacaagatggctgaggcgtactcggagattggtatgaagggcgagagacgtcgcggaaagggacacgacggcttataccaggggctttccaccgcgaccaaggacacatacgacgcgctgcacatgcaagccttaccacctcgatgaggtaccagcggccgcttcgagcagacatgataagatacattgatgagtttggacaaaccacaactagaatgcagtgaaaaaaatgctttatttgtgaaatttgtgatgctattgctttatttgtaaccattataagctgcaataaacaagttaacaacaacaattcgaatttaaatcggatccgcaacaaatctgactttgcatgtgcaaacgccttcaacaacagcattattccagaagacaccttcttccccagcccaggtaagggcagctttggtgccttcgcaggctgtttccttgcttcaggaatggccaggttctgcccagagctctggtcaatgatgtctaaaactcctctgattggtggtctcggccttatccattgccaccaaaaccctctttttactaagaaacagtgagccttgttctggcagtccagagaatgacacgggaaaaaagcagatgaagagaaggtggcaggagagggcacgtggcccagcctcagtctctccaactgagttcctgcctgcctgcctttgctcagactgtttgccccttactgctcttctaggcctcattctaagccccttctccaagttgcctctccttatttctccctgtctgccaaaaaatctttcccagctcactaagtcagtctcacgcagtcactcattaacccaccaatcactgattgtgccggcacatgaatgcaccaggtgttgaagtggaggaattaaaaagtcagatgaggggtgtgcccagaggaagcaccattctagttgggggagcccatctgtcagctgggaaaagtccaaataacttcagattggaatgtgttttaactcagggttgagaaaacagccaccttcaggacaaaagtcagggaagggctctctgaagaaatgctacttgaagataccagccctaccaagggcagggagaggaccaattgatggagttggccactccctctctgcgcgctcgctcgctcactgaggccgcccgggcaaagcccgggcgtcgggcgacctttggtcgcccggcctcagtgagcgagcgagcgcgcagagagggagtggccaacggcgcgcctgcaggtctcaaaaatagctaccctctccggcatgaatttatcagctagaacggttgaatatcatattgatggtgatttgactgtctccggcctttctcacccgtttgaatctttacctacacattactcaggcattgcatttaaaatatatgagggttctaaaaatttttatccttgcgttgaaataaaggcttctcccgcaaaagtattacagggtcataatgtttttggtacaaccgatttagctttatgctctgaggctttattgcttaattttgctaattctttgccttgcctgtatgatttattggatgttggaattcctgatgcggtattttctccttacgcatctgtgcggtatttcacaccgcatatggtgcactctcagtacaatctgctctgatgccgcatagttaagccagccccgacacccgccaacacccgctgacgcgccctgacgggcttgtctgctcccggcatccgcttacagacaagctgtgaccgtctccgggagctgcatgtgtcagaggttttcaccgtcatcaccgaaacgcgcgagacgaaagggcctcgtgatacgcctatttttataggttaatgtcatgataataatggtttcttagacgtcaggtggcacttttcggggaaatgtgcgcggaacccctatttgtttatttttctaaatacattcaaatatgtatccgctcatgagacaataaccctgataaatgcttcaataatattgaaaaaggaagagtatgagtattcaacatttccgtgtcgcccttattcccttttttgcggcattttgccttcctgtttttgctcacccagaaacgctggtgaaagtaaaagatgctgaagatcagttgggtgcacgagtgggttacatcgaactggatctcaacagcggtaagatccttgagagttttcgccccgaagaacgttttccaatgatgagcacttttaaagttctgctatgtggcgcggtattatcccgtattgacgccgggcaagagcaactcggtcgccgcatacactattctcagaatgacttggttgagtactcaccagtcacagaaaagcatcttacggatggcatgacagtaagagaattatgcagtgctgccataaccatgagtgataacactgcggccaacttacttctgacaacgatcggaggaccgaaggagctaaccgcttttttgcacaacatgggggatcatgtaactcgccttgatcgttgggaaccggagctgaatgaagccataccaaacgacgagcgtgacaccacgatgcctgtagcaatggcaacaacgttgcgcaaactattaactggcgaactacttactctagcttcccggcaacaattaatagactggatggaggcggataaagttgcaggaccacttctgcgctcggcccttccggctggctggtttattgctgataaatctggagccggtgagcgtgggtctcgcggtatcattgcagcactggggccagatggtaagccctcccgtatcgtagttatctacacgacggggagtcaggcaactatggatgaacgaaatagacagatcgctgagataggtgcctcactgattaagcattggtaactgtcagaccaagtttactcatatatactttagattgatttaaaacttcatttttaatttaaaaggatctaggtgaagatcctttttgataatctcatgaccaaaatcccttaacgtgagttttcgttccactgagcgtcagaccccgtagaaaagatcaaaggatcttcttgagatcctttttttctgcgcgtaatctgctgcttgcaaacaaaaaaaccaccgctaccagcggtggtttgtttgccggatcaagagctaccaactctttttccgaaggtaactggcttcagcagagcgcagataccaaatactgtccttctagtgtagccgtagttaggccaccacttcaagaactctgtagcaccgcctacatacctcgctctgctaatcctgttaccagtggctgctgccagtggcgataagtcgtgtcttaccgggttggactcaagacgatagttaccggataaggcgcagcggtcgggctgaacggggggttcgtgcacacagcccagcttggagcgaacgacctacaccgaactgagatacctacagcgtgagctatgagaaagcgccacgcttcccgaagggagaaaggcggacaggtatccggtaagcggcagggtcggaacaggagagcgcacgagggagcttccagggggaaacgcctggtatctttatagtcctgtcgggtttcgccacctctgacttgagcgtcgatttttgtgatgctcgtcaggggggcggagcctatggaaaaacgccagcaacgcggcctttttacggttcctggccttttgctggccttttgctcacatgttctttcctgcgttatcccctgattctgtggataaccgtattaccgcctttgagtgagctgataccgctcgccgcagccgaacgaccgagcgcagcgagtcagtgagcgaggaagcggaagagcgcccaatacgcaaaccgcctctccccgcgcgttggccgattcattaatg

SEQ ID NO: 30 - DNA, 7464 bp, Artificial Sequence
  Synthesized
cagcagctggcgtaatagcgaagaggcccgcaccgatcgcccttcccaacagttgcgcagcctgaatggcgaatggaattccagacgattgagcgtcaaaatgtaggtatttccatgagcgtttttcctgttgcaatggctggcggtaatattgttctggatattaccagcaaggccgatagtttgagttcttctactcaggcaagtgatgttattactaatcaaagaagtattgcgacaacggttaatttgcgtgatggacagactcttttactcggtggcctcactgattataaaaacacttctcaggattctggcgtaccgttcctgtctaaaatccctttaatcggcctcctgtttagctcccgctctgattctaacgaggaaagcacgttatacgtgctcgtcaaagcaaccatagtacgcgccctgtagcggcgcattaagcgcggcgggtgtggtggttacgcgcagcgtgaccgctacacttgccagcgccctagcgcccgctcctttcgctttcttcccttcctttctcgccacgttcgccggctttccccgtcaagctctaaatcgggggctccctttagggttccgatttagtgctttacggcacctcgaccccaaaaaacttgattagggtgatggttcacgtagtgggccatcgccctgatagacggtttttcgccctttgacgttggagtccacgttctttaatagtggactcttgttccaaactggaacaacactcaaccctatctcggtctattcttttgatttataagggattttgccgatttcggcctattggttaaaaaatgagctgatttaacaaaaatttaacgcgaattttaacaaaatattaacgtttacaatttaaatatttgcttatacaatcttcctgtttttggggcttttctgattatcaaccggggtacatatgattgacatgctagttttacggcgcgccgggttggccactccctctctgcgcgctcgctcgctcactgaggccgggcgaccaaaggtcgcccgacgcccgggctttgcccgggcggcctcagtgagcgagcgagcgcgcagagagggagtggccaactccatcactaggggttcctacgcgtagatctcatattctggcagggtcagtggctccaactaacatttgtttggtactttacagtttattaaatagatgtttatatggagaagctctcatttctttctcagaagagcctggctaggaaggtggatgaggcaccatattcattttgcaggtgaaattcctgagatgtaaggagctgctgtgacttgctcaaggccttatatcgagtaaacggtagcgctggggcttagacgcaggtgttctgatttatagttcaaaacctctatcaatgagagagcaatctcctggtaatgtgatagatttcccaacttaatgccaacataccataaacctcccattctgctaatgcccagcctaagttggggagaccactccagattccaagatgtacagtttgctttgctgggcctttttcccatgcctgcctttactctgccagagttatattgctggggttttgaagaagatcctattaaataaaagaataagcagtattattaagtagccctgcatttcaggtttccttgagtggcaggccaggcctggccgtgaacgttcactgaaatcatggcctcttggccaagattgatagcttgtgcctgtccctgagtcccagtccatcacgagcagctggtttctaagatgctatttcccgtataaagcatgagaccgtgacttgccagccccacagagccccgcccttgtccatcactggcatctggactccagcctgggttggggcaaagagggaaatgagatcatgtcctaaccctgatcctcttgtcccacagatatccagaaccctgaccctgccgtgtaccagctgagagactctaaatccagtgacaagtctgtctgcctattcaccgattttgattctcaaacaaatgtgtcacaaagtaaggattctgatgtgtatatcacagacaaaactgtgctagacatgaggtctatggacttcaagagcaacagtgctgtggcctggagcaactagtgggcggagttagggcggagccaatcagcgtgcgccgttccgaaagttgccttttatggctgggcggagaatgggcggtgaacgccgatgattatataaggacgcgccgggtgtggcacagctagttccgtcgcagccgggatttgggtcgcggttcttgtttgttccggaaagccaccatggcgctcccagtgacagccttacttttacctctggcgttattattgcacgcggctcgtcctgacatacagatgactcagactacctcttccctatctgcttctttaggcgaccgagtaacaatatcttgccgggccagccaggacatctcaaaatacttaaactggtatcagcagaagccggacggaacagttaagttgctcatttaccacacgtcgagattacactcaggcgttcctagccgattttcgggttccggttccggtacggactacagcctgacaatcagtaaccttgagcaggaggacatcgccacctacttctgtcagcagggcaacacgctcccgtacacattcggtgggggaactaagctggagattaccggaggcggtggcagcggtggcggcggcagcgggggtggcggctcggaggtcaagttacaggagagcggaccgggcttggtcgcacctagccagagcctctcagtcacgtgcactgtgtctggagtcagtctcccagactacggggtatcatggatacgacagccgcctagaaagggcttagagtggctgggggttatctggggaagtgaaaccacatactacaactcagctctcaagagccgcctcaccatcattaaggacaacagtaagtcgcaggttttcttaaagatgaactctctccagactgacgacaccgctatttactactgcgcgaagcactactactacggcgggagttacgcaatggactactggggtcagggcacttctgtgaccgtatccagcactactaccccagccccacgtccccccacgccagctccaacgatagcaagtcagcccttatctcttcgccctgaggcttgcaggcccgcggcgggcggcgccgttcacacgcgaggactagacttcgcctgcgacatctacatctgggcaccactagccgggacttgcggagtgttgttgttgagcttggtaataacgctctactgcaaacatagccgcaaaaaatttgtgcatctgctgaaacgcccgtttattaaaaccaccggcgcggcgcagatggaagatgcgagcagctgccgctgcccgcaggaagaagaaggcgaatgcgatctgagagtgaagttctctcgctccgcggacgcacccgcttaccagcagggtcagaaccagctatacaacgagttaaacctggggcgccgggaggagtacgacgtgttagacaagcgtagaggtagggacccggagatgggaggcaagcctcggagaaagaacccccaggagggcctgtacaacgaactccagaaggacaagatggctgaggcgtactcggagattggtatgaagggcgagagacgtcgcggaaagggacacgacggcttataccaggggctttccaccgcgaccaaggacacatacgacgcgctgcacatgcaagccttaccacctcgatgaggtaccagcggccgcttcgagcagacatgataagatacattgatgagtttggacaaaccacaactagaatgcagtgaaaaaaatgctttatttgtgaaatttgtgatgctattgctttatttgtaaccattataagctgcaataaacaagttaacaacaacaattcgaatttaaatcggatccgcaacaaatctgactttgcatgtgcaaacgccttcaacaacagcattattccagaagacaccttcttccccagcccaggtaagggcagctttggtgccttcgcaggctgtttccttgcttcaggaatggccaggttctgcccagagctctggtcaatgatgtctaaaactcctctgattggtggtctcggccttatccattgccaccaaaaccctctttttactaagaaacagtgagccttgttctggcagtccagagaatgacacgggaaaaaagcagatgaagagaaggtggcaggagagggcacgtggcccagcctcagtctctccaactgagttcctgcctgcctgcctttgctcagactgtttgccccttactgctcttctaggcctcattctaagccccttctccaagttgcctctccttatttctccctgtctgccaaaaaatctttcccagctcactaagtcagtctcacgcagtcactcattaacccaccaatcactgattgtgccggcacatgaatgcaccaggtgttgaagtggaggaattaaaaagtcagatgaggggtgtgcccagaggaagcaccattctagttgggggagcccatctgtcagctgggaaaagtccaaataacttcagattggaatgtgttttaactcagggttgagaaaacagccaccttcaggacaaaagtcagggaagggctctctgaagaaatgctacttgaagataccagccctaccaagggcagggagaggaccaattgatggagttggccactccctctctgcgcgctcgctcgctcactgaggccgcccgggcaaagcccgggcgtcgggcgacctttggtcgcccggcctcagtgagcgagcgagcgcgcagagagggagtggccaacggcgcgcctgcaggtctcaaaaatagctaccctctccggcatgaatttatcagctagaacggttgaatatcatattgatggtgatttgactgtctccggcctttctcacccgtttgaatctttacctacacattactcaggcattgcatttaaaatatatgagggttctaaaaatttttatccttgcgttgaaataaaggcttctcccgcaaaagtattacagggtcataatgtttttggtacaaccgatttagctttatgctctgaggctttattgcttaattttgctaattctttgccttgcctgtatgatttattggatgttggaattcctgatgcggtattttctccttacgcatctgtgcggtatttcacaccgcatatggtgcactctcagtacaatctgctctgatgccgcatagttaagccagccccgacacccgccaacacccgctgacgcgccctgacgggcttgtctgctcccggcatccgcttacagacaagctgtgaccgtctccgggagctgcatgtgtcagaggttttcaccgtcatcaccgaaacgcgcgagacgaaagggcctcgtgatacgcctatttttataggttaatgtcatgataataatggtttcttagacgtcaggtggcacttttcggggaaatgtgcgcggaacccctatttgtttatttttctaaatacattcaaatatgtatccgctcatgagacaataaccctgataaatgcttcaataatattgaaaaaggaagagtatgagtattcaacatttccgtgtcgcccttattcccttttttgcggcattttgccttcctgtttttgctcacccagaaacgctggtgaaagtaaaagatgctgaagatcagttgggtgcacgagtgggttacatcgaactggatctcaacagcggtaagatccttgagagttttcgccccgaagaacgttttccaatgatgagcacttttaaagttctgctatgtggcgcggtattatcccgtattgacgccgggcaagagcaactcggtcgccgcatacactattctcagaatgacttggttgagtactcaccagtcacagaaaagcatcttacggatggcatgacagtaagagaattatgcagtgctgccataaccatgagtgataacactgcggccaacttacttctgacaacgatcggaggaccgaaggagctaaccgcttttttgcacaacatgggggatcatgtaactcgccttgatcgttgggaaccggagctgaatgaagccataccaaacgacgagcgtgacaccacgatgcctgtagcaatggcaacaacgttgcgcaaactattaactggcgaactacttactctagcttcccggcaacaattaatagactggatggaggcggataaagttgcaggaccacttctgcgctcggcccttccggctggctggtttattgctgataaatctggagccggtgagcgtgggtctcgcggtatcattgcagcactggggccagatggtaagccctcccgtatcgtagttatctacacgacggggagtcaggcaactatggatgaacgaaatagacagatcgctgagataggtgcctcactgattaagcattggtaactgtcagaccaagtttactcatatatactttagattgatttaaaacttcatttttaatttaaaaggatctaggtgaagatcctttttgataatctcatgaccaaaatcccttaacgtgagttttcgttccactgagcgtcagaccccgtagaaaagatcaaaggatcttcttgagatcctttttttctgcgcgtaatctgctgcttgcaaacaaaaaaaccaccgctaccagcggtggtttgtttgccggatcaagagctaccaactctttttccgaaggtaactggcttcagcagagcgcagataccaaatactgtccttctagtgtagccgtagttaggccaccacttcaagaactctgtagcaccgcctacatacctcgctctgctaatcctgttaccagtggctgctgccagtggcgataagtcgtgtcttaccgggttggactcaagacgatagttaccggataaggcgcagcggtcgggctgaacggggggttcgtgcacacagcccagcttggagcgaacgacctacaccgaactgagatacctacagcgtgagctatgagaaagcgccacgcttcccgaagggagaaaggcggacaggtatccggtaagcggcagggtcggaacaggagagcgcacgagggagcttccagggggaaacgcctggtatctttatagtcctgtcgggtttcgccacctctgacttgagcgtcgatttttgtgatgctcgtcaggggggcggagcctatggaaaaacgccagcaacgcggcctttttacggttcctggccttttgctggccttttgctcacatgttctttcctgcgttatcccctgattctgtggataaccgtattaccgcctttgagtgagctgataccgctcgccgcagccgaacgaccgagcgcagcgagtcagtgagcgaggaagcggaagagcgcccaatacgcaaaccgcctctccccgcgcgttggccgattcattaatg

SEQ ID NO: 31 - DNA, 7464 bp, Artificial Sequence
  Synthesized
cagcagctggcgtaatagcgaagaggcccgcaccgatcgcccttcccaacagttgcgcagcctgaatggcgaatggaattccagacgattgagcgtcaaaatgtaggtatttccatgagcgtttttcctgttgcaatggctggcggtaatattgttctggatattaccagcaaggccgatagtttgagttcttctactcaggcaagtgatgttattactaatcaaagaagtattgcgacaacggttaatttgcgtgatggacagactcttttactcggtggcctcactgattataaaaacacttctcaggattctggcgtaccgttcctgtctaaaatccctttaatcggcctcctgtttagctcccgctctgattctaacgaggaaagcacgttatacgtgctcgtcaaagcaaccatagtacgcgccctgtagcggcgcattaagcgcggcgggtgtggtggttacgcgcagcgtgaccgctacacttgccagcgccctagcgcccgctcctttcgctttcttcccttcctttctcgccacgttcgccggctttccccgtcaagctctaaatcgggggctccctttagggttccgatttagtgctttacggcacctcgaccccaaaaaacttgattagggtgatggttcacgtagtgggccatcgccctgatagacggtttttcgccctttgacgttggagtccacgttctttaatagtggactcttgttccaaactggaacaacactcaaccctatctcggtctattcttttgatttataagggattttgccgatttcggcctattggttaaaaaatgagctgatttaacaaaaatttaacgcgaattttaacaaaatattaacgtttacaatttaaatatttgcttatacaatcttcctgtttttggggcttttctgattatcaaccggggtacatatgattgacatgctagttttacggcgcgccgggttggccactccctctctgcgcgctcgctcgctcactgaggccgggcgaccaaaggtcgcccgacgcccgggctttgcccgggcggcctcagtgagcgagcgagcgcgcagagagggagtggccaactccatcactaggggttcctacgcgtagatctcatattctggcagggtcagtggctccaactaacatttgtttggtactttacagtttattaaatagatgtttatatggagaagctctcatttctttctcagaagagcctggctaggaaggtggatgaggcaccatattcattttgcaggtgaaattcctgagatgtaaggagctgctgtgacttgctcaaggccttatatcgagtaaacggtagcgctggggcttagacgcaggtgttctgatttatagttcaaaacctctatcaatgagagagcaatctcctggtaatgtgatagatttcccaacttaatgccaacataccataaacctcccattctgctaatgcccagcctaagttggggagaccactccagattccaagatgtacagtttgctttgctgggcctttttcccatgcctgcctttactctgccagagttatattgctggggttttgaagaagatcctattaaataaaagaataagcagtattattaagtagccctgcatttcaggtttccttgagtggcaggccaggcctggccgtgaacgttcactgaaatcatggcctcttggccaagattgatagcttgtgcctgtccctgagtcccagtccatcacgagcagctggtttctaagatgctatttcccgtataaagcatgagaccgtgacttgccagccccacagagccccgcccttgtccatcactggcatctggactccagcctgggttggggcaaagagggaaatgagatcatgtcctaaccctgatcctcttgtcccacagatatccagaaccctgaccctgccgtgtaccagctgagagactctaaatccagtgacaagtctgtctgcctattcaccgattttgattctcaaacaaatgtgtcacaaagtaaggattctgatgtgtatatcacagacaaaactgtgctagacatgaggtctatggacttcaagagcaacagtgctgtggcctggagcaactagtgggcggagttagggcggagccaatcagcgtgcgccgttccgaaagttgccttttatggctgggcggagaatgggcggtgaacgccgatgattatataaggacgcgccgggtgtggcacagctagttccgtcgcagccgggatttgggtcgcggttcttgtttgttccggaaagccaccatggcgctcccagtgacagccttacttttacctctggcgttattattgcacgcggctcgtcctgacatacagatgactcagactacctcttccctatctgcttctttaggcgaccgagtaacaatatcttgccgggccagccaggacatctcaaaatacttaaactggtatcagcagaagccggacggaacagttaagttgctcatttaccacacgtcgagattacactcaggcgttcctagccgattttcgggttccggttccggtacggactacagcctgacaatcagtaaccttgagcaggaggacatcgccacctacttctgtcagcagggcaacacgctcccgtacacattcggtgggggaactaagctggagattaccggaggcggtggcagcggtggcggcggcagcgggggtggcggctcggaggtcaagttacaggagagcggaccgggcttggtcgcacctagccagagcctctcagtcacgtgcactgtgtctggagtcagtctcccagactacggggtatcatggatacgacagccgcctagaaagggcttagagtggctgggggttatctggggaagtgaaaccacatactacaactcagctctcaagagccgcctcaccatcattaaggacaacagtaagtcgcaggttttcttaaagatgaactctctccagactgacgacaccgctatttactactgcgcgaagcactactactacggcgggagttacgcaatggactactggggtcagggcacttctgtgaccgtatccagcactactaccccagccccacgtccccccacgccagctccaacgatagcaagtcagcccttatctcttcgccctgaggcttgcaggcccgcggcgggcggcgccgttcacacgcgaggactagacttcgcctgcgacatctacatctgggcaccactagccgggacttgcggagtgttgttgttgagcttggtaataacgctctactgcaaagcgagccgcaaaaaagcggcggcggcggcgaaaagcccgtttgcgagcccggcgagcagcgcgcaggaagaagatgcgagcagctgccgcgcgccgagcgaagaagaaggcagctgcgaactgagagtgaagttctctcgctccgcggacgcacccgcttaccagcagggtcagaaccagctatacaacgagttaaacctggggcgccgggaggagtacgacgtgttagacaagcgtagaggtagggacccggagatgggaggcaagcctcggagaaagaacccccaggagggcctgtacaacgaactccagaaggacaagatggctgaggcgtactcggagattggtatgaagggcgagagacgtcgcggaaagggacacgacggcttataccaggggctttccaccgcgaccaaggacacatacgacgcgctgcacatgcaagccttaccacctcgatgaggtaccagcggccgcttcgagcagacatgataagatacattgatgagtttggacaaaccacaactagaatgcagtgaaaaaaatgctttatttgtgaaatttgtgatgctattgctttatttgtaaccattataagctgcaataaacaagttaacaacaacaattcgaatttaaatcggatccgcaacaaatctgactttgcatgtgcaaacgccttcaacaacagcattattccagaagacaccttcttccccagcccaggtaagggcagctttggtgccttcgcaggctgtttccttgcttcaggaatggccaggttctgcccagagctctggtcaatgatgtctaaaactcctctgattggtggtctcggccttatccattgccaccaaaaccctctttttactaagaaacagtgagccttgttctggcagtccagagaatgacacgggaaaaaagcagatgaagagaaggtggcaggagagggcacgtggcccagcctcagtctctccaactgagttcctgcctgcctgcctttgctcagactgtttgccccttactgctcttctaggcctcattctaagccccttctccaagttgcctctccttatttctccctgtctgccaaaaaatctttcccagctcactaagtcagtctcacgcagtcactcattaacccaccaatcactgattgtgccggcacatgaatgcaccaggtgttgaagtggaggaattaaaaagtcagatgaggggtgtgcccagaggaagcaccattctagttgggggagcccatctgtcagctgggaaaagtccaaataacttcagattggaatgtgttttaactcagggttgagaaaacagccaccttcaggacaaaagtcagggaagggctctctgaagaaatgctacttgaagataccagccctaccaagggcagggagaggaccaattgatggagttggccactccctctctgcgcgctcgctcgctcactgaggccgcccgggcaaagcccgggcgtcgggcgacctttggtcgcccggcctcagtgagcgagcgagcgcgcagagagggagtggccaacggcgcgcctgcaggtctcaaaaatagctaccctctccggcatgaatttatcagctagaacggttgaatatcatattgatggtgatttgactgtctccggcctttctcacccgtttgaatctttacctacacattactcaggcattgcatttaaaatatatgagggttctaaaaatttttatccttgcgttgaaataaaggcttctcccgcaaaagtattacagggtcataatgtttttggtacaaccgatttagctttatgctctgaggctttattgcttaattttgctaattctttgccttgcctgtatgatttattggatgttggaattcctgatgcggtattttctccttacgcatctgtgcggtatttcacaccgcatatggtgcactctcagtacaatctgctctgatgccgcatagttaagccagccccgacacccgccaacacccgctgacgcgccctgacgggcttgtctgctcccggcatccgcttacagacaagctgtgaccgtctccgggagctgcatgtgtcagaggttttcaccgtcatcaccgaaacgcgcgagacgaaagggcctcgtgatacgcctatttttataggttaatgtcatgataataatggtttcttagacgtcaggtggcacttttcggggaaatgtgcgcggaacccctatttgtttatttttctaaatacattcaaatatgtatccgctcatgagacaataaccctgataaatgcttcaataatattgaaaaaggaagagtatgagtattcaacatttccgtgtcgcccttattcccttttttgcggcattttgccttcctgtttttgctcacccagaaacgctggtgaaagtaaaagatgctgaagatcagttgggtgcacgagtgggttacatcgaactggatctcaacagcggtaagatccttgagagttttcgccccgaagaacgttttccaatgatgagcacttttaaagttctgctatgtggcgcggtattatcccgtattgacgccgggcaagagcaactcggtcgccgcatacactattctcagaatgacttggttgagtactcaccagtcacagaaaagcatcttacggatggcatgacagtaagagaattatgcagtgctgccataaccatgagtgataacactgcggccaacttacttctgacaacgatcggaggaccgaaggagctaaccgcttttttgcacaacatgggggatcatgtaactcgccttgatcgttgggaaccggagctgaatgaagccataccaaacgacgagcgtgacaccacgatgcctgtagcaatggcaacaacgttgcgcaaactattaactggcgaactacttactctagcttcccggcaacaattaatagactggatggaggcggataaagttgcaggaccacttctgcgctcggcccttccggctggctggtttattgctgataaatctggagccggtgagcgtgggtctcgcggtatcattgcagcactggggccagatggtaagccctcccgtatcgtagttatctacacgacggggagtcaggcaactatggatgaacgaaatagacagatcgctgagataggtgcctcactgattaagcattggtaactgtcagaccaagtttactcatatatactttagattgatttaaaacttcatttttaatttaaaaggatctaggtgaagatcctttttgataatctcatgaccaaaatcccttaacgtgagttttcgttccactgagcgtcagaccccgtagaaaagatcaaaggatcttcttgagatcctttttttctgcgcgtaatctgctgcttgcaaacaaaaaaaccaccgctaccagcggtggtttgtttgccggatcaagagctaccaactctttttccgaaggtaactggcttcagcagagcgcagataccaaatactgtccttctagtgtagccgtagttaggccaccacttcaagaactctgtagcaccgcctacatacctcgctctgctaatcctgttaccagtggctgctgccagtggcgataagtcgtgtcttaccgggttggactcaagacgatagttaccggataaggcgcagcggtcgggctgaacggggggttcgtgcacacagcccagcttggagcgaacgacctacaccgaactgagatacctacagcgtgagctatgagaaagcgccacgcttcccgaagggagaaaggcggacaggtatccggtaagcggcagggtcggaacaggagagcgcacgagggagcttccagggggaaacgcctggtatctttatagtcctgtcgggtttcgccacctctgacttgagcgtcgatttttgtgatgctcgtcaggggggcggagcctatggaaaaacgccagcaacgcggcctttttacggttcctggccttttgctggccttttgctcacatgttctttcctgcgttatcccctgattctgtggataaccgtattaccgcctttgagtgagctgataccgctcgccgcagccgaacgaccgagcgcagcgagtcagtgagcgaggaagcggaagagcgcccaatacgcaaaccgcctctccccgcgcgttggccgattcattaatg

SEQ ID NO: 32 - DNA, 164 bp, Artificial Sequence
  Synthesized
gggcggagttagggcggagccaatcagcgtgcgccgttccgaaagttgccttttatggctgggcggagaatgggcggtgaacgccgatgattatataaggacgcgccgggtgtggcacagctagttccgtcgcagccgggatttgggtcgcggttcttgtttgt

SEQ ID NO: 33 - DNA, 122 bp, Artificial Sequence
  Synthesized
taagatacattgatgagtttggacaaaccacaactagaatgcagtgaaaaaaatgctttatttgtgaaatttgtgatgctattgctttatttgtaaccattataagctgcaataaacaagtt

SEQ ID NO: 34 - DNA, 135 bp, Artificial Sequence
  Synthesized
gatccagacatgataagatacattgatgagtttggacaaaccacaactagaatgcagtgaaaaaaatgctttatttgtgaaatttgtgatgctattgctttatttgtaaccattataagctgcaataaacaagtt

SEQ ID NO: 35 - DNA, 181 bp, Artificial Sequence
  Synthesized
tgagtttggacaaaccacaactagaatgcagtgaaaaaaatgctttatttgtgaaatttgtgatgctattgctttatttgtaaccattataagctgcaataaacaagttaacaacaacaattgcattcattttatgtttcaggttcagggggaggtgtgggaggttttttaaagcaagtaa

SEQ ID NO: 36 - DNA, 7521 bp, Artificial Sequence
  Synthesized
cagcagctggcgtaatagcgaagaggcccgcaccgatcgcccttcccaacagttgcgcagcctgaatggcgaatggaattccagacgattgagcgtcaaaatgtaggtatttccatgagcgtttttcctgttgcaatggctggcggtaatattgttctggatattaccagcaaggccgatagtttgagttcttctactcaggcaagtgatgttattactaatcaaagaagtattgcgacaacggttaatttgcgtgatggacagactcttttactcggtggcctcactgattataaaaacacttctcaggattctggcgtaccgttcctgtctaaaatccctttaatcggcctcctgtttagctcccgctctgattctaacgaggaaagcacgttatacgtgctcgtcaaagcaaccatagtacgcgccctgtagcggcgcattaagcgcggcgggtgtggtggttacgcgcagcgtgaccgctacacttgccagcgccctagcgcccgctcctttcgctttcttcccttcctttctcgccacgttcgccggctttccccgtcaagctctaaatcgggggctccctttagggttccgatttagtgctttacggcacctcgaccccaaaaaacttgattagggtgatggttcacgtagtgggccatcgccctgatagacggtttttcgccctttgacgttggagtccacgttctttaatagtggactcttgttccaaactggaacaacactcaaccctatctcggtctattcttttgatttataagggattttgccgatttcggcctattggttaaaaaatgagctgatttaacaaaaatttaacgcgaattttaacaaaatattaacgcttacaatttaaatatttgcttatacaatcttcctgtttttggggcttttctgattatcaaccggggtacatatgattgacatgctagttttacggcgcgccgggttggccactccctctctgcgcgctcgctcgctcactgaggccgggcgaccaaaggtcgcccgacgcccgggctttgcccgggcggcctcagtgagcgagcgagcgcgcagagagggagtggccaactccatcactaggggttcctacgcgtagatctcatattctggcagggtcagtggctccaactaacatttgtttggtactttacagtttattaaatagatgtttatatggagaagctctcatttctttctcagaagagcctggctaggaaggtggatgaggcaccatattcattttgcaggtgaaattcctgagatgtaaggagctgctgtgacttgctcaaggccttatatcgagtaaacggtagcgctggggcttagacgcaggtgttctgatttatagttcaaaacctctatcaatgagagagcaatctcctggtaatgtgatagatttcccaacttaatgccaacataccataaacctcccattctgctaatgcccagcctaagttggggagaccactccagattccaagatgtacagtttgctttgctgggcctttttcccatgcctgcctttactctgccagagttatattgctggggttttgaagaagatcctattaaataaaagaataagcagtattattaagtagccctgcatttcaggtttccttgagtggcaggccaggcctggccgtgaacgttcactgaaatcatggcctcttggccaagattgatagcttgtgcctgtccctgagtcccagtccatcacgagcagctggtttctaagatgctatttcccgtataaagcatgagaccgtgacttgccagccccacagagccccgcccttgtccatcactggcatctggactccagcctgggttggggcaaagagggaaatgagatcatgtcctaaccctgatcctcttgtcccacagatatccagaaccctgaccctgccgtgtaccagctgagagactctaaatccagtgacaagtctgtctgcctattcaccgattttgattctcaaacaaatgtgtcacaaagtaaggattctgatgtgtatatcacagacaaaactgtgctagacatgaggtctatggacttcaagagcaacagtgctgtggcctggagcaactagtgggcggagttagggcggagccaatcagcgtgcgccgttccgaaagttgccttttatggctgggcggagaatgggcggtgaacgccgatgattatataaggacgcgccgggtgtggcacagctagttccgtcgcagccgggatttgggtcgcggttcttgtttgttccggaaagccacatggcgctcccagtgacagccttacttttacctctggcgttattattgcacgcggctcgtcctgacatacagatgactcagactacctcttccctatctgcttctttaggcgaccgagtaacaatatcttgccgggccagccaggacatctcaaaatacttaaactggtatcagcagaagccggacggaacagttaagttgctcatttaccacacgtcgagattacactcaggcgttcctagccgattttcgggttccggttccggtacggactacagcctgacaatcagtaaccttgagcaggaggacatcgccacctacttctgtcagcagggcaacacgctcccgtacacattcggtgggggaactaagctggagattaccggaggcggtggcagcggtggcggcggcagcgggggtggcggctcggaggtcaagttacaggagagcggaccgggcttggtcgcacctagccagagcctctcagtcacgtgcactgtgtctggagtcagtctcccagactacggggtatcatggatacgacagccgcctagaaagggcttagagtggctgggggttatctggggaagtgaaaccacatactacaactcagctctcaagagccgcctcaccatcattaaggacaacagtaagtcgcaggttttcttaaagatgaactctctccagactgacgacaccgctatttactactgcgcgaagcactactactacggcgggagttacgcaatggactactggggtcagggcacttctgtgaccgtatccagcactactaccccagccccacgtccccccacgccagctccaacgatagcaagtcagcccttatctcttcgccctgaggcttgcaggcccgcggcgggcggcgccgttcacacgcgaggactagacttcgcctgcgacatctacatctgggcaccactagccgggacttgcggagtgttgttgttgagcttggtaataacgctctactgcaagcgtgggagaaagaagctcttgtacattttcaagcagccattcatgcgtcccgttcagacgactcaggaggaggacggctgctcgtgccgattcccggaggaggaggagggcggttgcgaactcagagtgaagttctctcgctccgcggacgcacccgcttaccagcagggtcagaaccagctatacaacgagttaaacctggggcgccgggaggagtacgacgtgttagacaagcgtagaggtagggacccggagatgggaggcaagcctcggagaaagaacccccaggagggcctgtacaacgaactccagaaggacaagatggctgaggcgtactcggagattggtatgaagggcgagagacgtcgcggaaagggacacgacggcttataccaggggctttccaccgcgaccaaggacacatacgacgcgctgcacatgcaagccttaccacctcgatgaggtaccagcggccgcgatccagacatgataagatacattgatgagtttggacaaaccacaactagaatgcagtgaaaaaaatgctttatttgtgaaatttgtgatgctattgctttatttgtaaccattataagctgcaataaacaagttaacaacaacaattgcattcattttatgtttcaggttcagggggaggtgtgggaggttttttaaagcaagtaaactggtactagtacggatccgcaacaaatctgactttgcatgtgcaaacgccttcaacaacagcattattccagaagacaccttcttccccagcccaggtaagggcagctttggtgccttcgcaggctgtttccttgcttcaggaatggccaggttctgcccagagctctggtcaatgatgtctaaaactcctctgattggtggtctcggccttatccattgccaccaaaaccctctttttactaagaaacagtgagccttgttctggcagtccagagaatgacacgggaaaaaagcagatgaagagaaggtggcaggagagggcacgtggcccagcctcagtctctccaactgagttcctgcctgcctgcctttgctcagactgtttgccccttactgctcttctaggcctcattctaagccccttctccaagttgcctctccttatttctccctgtctgccaaaaaatctttcccagctcactaagtcagtctcacgcagtcactcattaacccaccaatcactgattgtgccggcacatgaatgcaccaggtgttgaagtggaggaattaaaaagtcagatgaggggtgtgcccagaggaagcaccattctagttgggggagcccatctgtcagctgggaaaagtccaaataacttcagattggaatgtgttttaactcagggttgagaaaacagccaccttcaggacaaaagtcagggaagggctctctgaagaaatgctacttgaagataccagccctaccaagggcagggagaggaccaattgatggagttggccactccctctctgcgcgctcgctcgctcactgaggccgcccgggcaaagcccgggcgtcgggcgacctttggtcgcccggcctcagtgagcgagcgagcgcgcagagagggagtggccaacggcgcgcctgcaggttcaaaaatagctaccctctccggcatgaatttatcagctagaacggttgaatatcatattgatggtgatttgactgtctccggcctttctcacccgtttgaatctttacctacacattactcaggcattgcatttaaaatatatgagggttctaaaaatttttatccttgcgttgaaataaaggcttctcccgcaaaagtattacagggtcataatgtttttggtacaaccgatttagctttatgctctgaggctttattgcttaattttgctaattctttgccttgcctgtatgatttattggatgttggaattcctgatgcggtattttctccttacgcatctgtgcggtatttcacaccgcatatggtgcactctcagtacaatctgctctgatgccgcatagttaagccagccccgacacccgccaacacccgctgacgcgccctgacgggcttgtctgctcccggcatccgcttacagacaagctgtgaccgtctccgggagctgcatgtgtcagaggttttcaccgtcatcaccgaaacgcgcgagacgaaagggcctcgtgatacgcctatttttataggttaatgtcatgataataatggtttcttagacgtcaggtggcacttttcggggaaatgtgcgcggaacccctatttgtttatttttctaaatacattcaaatatgtatccgctcatgagacaataaccctgataaatgcttcaataatattgaaaaaggaagagtatgagtattcaacatttccgtgtcgcccttattcccttttttgcggcattttgccttcctgtttttgctcacccagaaacgctggtgaaagtaaaagatgctgaagatcagttgggtgcacgagtgggttacatcgaactggatctcaacagcggtaagatccttgagagttttcgccccgaagaacgttttccaatgatgagcacttttaaagttctgctatgtggcgcggtattatcccgtattgacgccgggcaagagcaactcggtcgccgcatacactattctcagaatgacttggttgagtactcaccagtcacagaaaagcatcttacggatggcatgacagtaagagaattatgcagtgctgccataaccatgagtgataacactgcggccaacttacttctgacaacgatcggaggaccgaaggagctaaccgcttttttgcacaacatgggggatcatgtaactcgccttgatcgttgggaaccggagctgaatgaagccataccaaacgacgagcgtgacaccacgatgcctgtagcaatggcaacaacgttgcgcaaactattaactggcgaactacttactctagcttcccggcaacaattaatagactggatggaggcggataaagttgcaggaccacttctgcgctcggcccttccggctggctggtttattgctgataaatctggagccggtgagcgtgggtctcgcggtatcattgcagcactggggccagatggtaagccctcccgtatcgtagttatctacacgacggggagtcaggcaactatggatgaacgaaatagacagatcgctgagataggtgcctcactgattaagcattggtaactgtcagaccaagtttactcatatatactttagattgatttaaaacttcatttttaatttaaaaggatctaggtgaagatcctttttgataatctcatgaccaaaatcccttaacgtgagttttcgttccactgagcgtcagaccccgtagaaaagatcaaaggatcttcttgagatcctttttttctgcgcgtaatctgctgcttgcaaacaaaaaaaccaccgctaccagcggtggtttgtttgccggatcaagagctaccaactctttttccgaaggtaactggcttcagcagagcgcagataccaaatactgtccttctagtgtagccgtagttaggccaccacttcaagaactctgtagcaccgcctacatacctcgctctgctaatcctgttaccagtggctgctgccagtggcgataagtcgtgtcttaccgggttggactcaagacgatagttaccggataaggcgcagcggtcgggctgaacggggggttcgtgcacacagcccagcttggagcgaacgacctacaccgaactgagatacctacagcgtgagctatgagaaagcgccacgcttcccgaagggagaaaggcggacaggtatccggtaagcggcagggtcggaacaggagagcgcacgagggagcttccagggggaaacgcctggtatctttatagtcctgtcgggtttcgccacctctgacttgagcgtcgatttttgtgatgctcgtcaggggggcggagcctatggaaaaacgccagcaacgcggcctttttacggttcctggccttttgctggccttttgctcacatgttctttcctgcgttatcccctgattctgtggataaccgtattaccgcctttgagtgagctgataccgctcgccgcagccgaacgaccgagcgcagcgagtcagtgagcgaggaagcggaagagcgcccaatacgcaaaccgcctctccccgcgcgttggccgattcattaatg

SEQ ID NO: 37 - DNA, 7464 bp, Artificial Sequence; identical to SEQ ID NO: 31
  Synthesized

SEQ ID NO: 38 - DNA, 7523 bp, Artificial Sequence
  Synthesized
cagcagctggcgtaatagcgaagaggcccgcaccgatcgcccttcccaacagttgcgcagcctgaatggcgaatggaattccagacgattgagcgtcaaaatgtaggtatttccatgagcgtttttcctgttgcaatggctggcggtaatattgttctggatattaccagcaaggccgatagtttgagttcttctactcaggcaagtgatgttattactaatcaaagaagtattgcgacaacggttaatttgcgtgatggacagactcttttactcggtggcctcactgattataaaaacacttctcaggattctggcgtaccgttcctgtctaaaatccctttaatcggcctcctgtttagctcccgctctgattctaacgaggaaagcacgttatacgtgctcgtcaaagcaaccatagtacgcgccctgtagcggcgcattaagcgcggcgggtgtggtggttacgcgcagcgtgaccgctacacttgccagcgccctagcgcccgctcctttcgctttcttcccttcctttctcgccacgttcgccggctttccccgtcaagctctaaatcgggggctccctttagggttccgatttagtgctttacggcacctcgaccccaaaaaacttgattagggtgatggttcacgtagtgggccatcgccctgatagacggtttttcgccctttgacgttggagtccacgttctttaatagtggactcttgttccaaactggaacaacactcaaccctatctcggtctattcttttgatttataagggattttgccgatttcggcctattggttaaaaaatgagctgatttaacaaaaatttaacgcgaattttaacaaaatattaacgtttacaatttaaatatttgcttatacaatcttcctgtttttggggcttttctgattatcaaccggggtacatatgattgacatgctagttttacggcgcgccgggttggccactccctctctgcgcgctcgctcgctcactgaggccgggcgaccaaaggtcgcccgacgcccgggctttgcccgggcggcctcagtgagcgagcgagcgcgcagagagggagtggccaactccatcactaggggttcctacgcgtagatctcatattctggcagggtcagtggctccaactaacatttgtttggtactttacagtttattaaatagatgtttatatggagaagctctcatttctttctcagaagagcctggctaggaaggtggatgaggcaccatattcattttgcaggtgaaattcctgagatgtaaggagctgctgtgacttgctcaaggccttatatcgagtaaacggtagcgctggggcttagacgcaggtgttctgatttatagttcaaaacctctatcaatgagagagcaatctcctggtaatgtgatagatttcccaacttaatgccaacataccataaacctcccattctgctaatgcccagcctaagttggggagaccactccagattccaagatgtacagtttgctttgctgggcctttttcccatgcctgcctttactctgccagagttatattgctggggttttgaagaagatcctattaaataaaagaataagcagtattattaagtagccctgcatttcaggtttccttgagtggcaggccaggcctggccgtgaacgttcactgaaatcatggcctcttggccaagattgatagcttgtgcctgtccctgagtcccagtccatcacgagcagctggtttctaagatgctatttcccgtataaagcatgagaccgtgacttgccagccccacagagccccgcccttgtccatcactggcatctggactccagcctgggttggggcaaagagggaaatgagatcatgtcctaaccctgatcctcttgtcccacagatatccagaaccctgaccctgccgtgtaccagctgagagactctaaatccagtgacaagtctgtctgcctattcaccgattttgattctcaaacaaatgtgtcacaaagtaaggattctgatgtgtatatcacagacaaaactgtgctagacatgaggtctatggacttcaagagcaacagtgctgtggcctggagcaactagtgggcggagttagggcggagccaatcagcgtgcgccgttccgaaagttgccttttatggctgggcggagaatgggcggtgaacgccgatgattatataaggacgcgccgggtgtggcacagctagttccgtcgcagccgggatttgggtcgcggttcttgtttgttccggaaagccaccatggcgctcccagtgacagccttacttttacctctggcgttattattgcacgcggctcgtcctgacatacagatgactcagactacctcttccctatctgcttctttaggcgaccgagtaacaatatcttgccgggccagccaggacatctcaaaatacttaaactggtatcagcagaagccggacggaacagttaagttgctcatttaccacacgtcgagattacactcaggcgttcctagccgattttcgggttccggttccggtacggactacagcctgacaatcagtaaccttgagcaggaggacatcgccacctacttctgtcagcagggcaacacgctcccgtacacattcggtgggggaactaagctggagattaccggaggcggtggcagcggtggcggcggcagcgggggtggcggctcggaggtcaagttacaggagagcggaccgggcttggtcgcacctagccagagcctctcagtcacgtgcactgtgtctggagtcagtctcccagactacggggtatcatggatacgacagccgcctagaaagggcttagagtggctgggggttatctggggaagtgaaaccacatactacaactcagctctcaagagccgcctcaccatcattaaggacaacagtaagtcgcaggttttcttaaagatgaactctctccagactgacgacaccgctatttactactgcgcgaagcactactactacggcgggagttacgcaatggactactggggtcagggcacttctgtgaccgtatccagcactactaccccagccccacgtccccccacgccagctccaacgatagcaagtcagcccttatctcttcgccctgaggcttgcaggcccgcggcgggcggcgccgttcacacgcgaggactagacttcgcctgcgacatctacatctgggcaccactagccgggacttgcggagtgttgttgttgagcttggtaataacgctctactgcaaagcgagccgcaaaaaagcggcggcggcggcgaaaagcccgtttgcgagcccggcgagcagcgcgcaggaagaagatgcgagcagctgccgcgcgccgagcgaagaagaaggcagctgcgaactgagagtgaagttctctcgctccgcggacgcacccgcttaccagcagggtcagaaccagctatacaacgagttaaacctggggcgccgggaggagtacgacgtgttagacaagcgtagaggtagggacccggagatgggaggcaagcctcggagaaagaacccccaggagggcctgtacaacgaactccagaaggacaagatggctgaggcgtactcggagattggtatgaagggcgagagacgtcgcggaaagggacacgacggcttataccaggggctttccaccgcgaccaaggacacatacgacgcgctgcacatgcaagccttaccacctcgatgaggtaccagcggccgcgatccagacatgataagatacattgatgagtttggacaaaccacaactagaatgcagtgaaaaaaatgctttatttgtgaaatttgtgatgctattgctttatttgtaaccattataagctgcaataaacaagttaacaacaacaattgcattcattttatgtttcaggttcagggggaggtgtgggaggttttttaaagcaagtaaactggtactagtacggatccgcaacaaatctgactttgcatgtgcaaacgccttcaacaacagcattattccagaagacaccttcttccccagcccaggtaagggcagctttggtgccttcgcaggctgtttccttgcttcaggaatggccaggttctgcccagagctctggtcaatgatgtctaaaactcctctgattggtggtctcggccttatccattgccaccaaaaccctctttttactaagaaacagtgagccttgttctggcagtccagagaatgacacgggaaaaaagcagatgaagagaaggtggcaggagagggcacgtggcccagcctcagtctctccaactgagttcctgcctgcctgcctttgctcagactgtttgccccttactgctcttctaggcctcattctaagccccttctccaagttgcctctccttatttctccctgtctgccaaaaaatctttcccagctcactaagtcagtctcacgcagtcactcattaacccaccaatcactgattgtgccggcacatgaatgcaccaggtgttgaagtggaggaattaaaaagtcagatgaggggtgtgcccagaggaagcaccattctagttgggggagcccatctgtcagctgggaaaagtccaaataacttcagattggaatgtgttttaactcagggttgagaaaacagccaccttcaggacaaaagtcagggaagggctctctgaagaaatgctacttgaagataccagccctaccaagggcagggagaggaccaattgatggagttggccactccctctctgcgcgctcgctcgctcactgaggccgcccgggcaaagcccgggcgtcgggcgacctttggtcgcccggcctcagtgagcgagcgagcgcgcagagagggagtggccaacggcgcgcctgcaggtctcaaaaatagctaccctctccggcatgaatttatcagctagaacggttgaatatcatattgatggtgatttgactgtctccggcctttctcacccgtttgaatctttacctacacattactcaggcattgcatttaaaatatatgagggttctaaaaatttttatccttgcgttgaaataaaggcttctcccgcaaaagtattacagggtcataatgtttttggtacaaccgatttagctttatgctctgaggctttattgcttaattttgctaattctttgccttgcctgtatgatttattggatgttggaattcctgatgcggtattttctccttacgcatctgtgcggtatttcacaccgcatatggtgcactctcagtacaatctgctctgatgccgcatagttaagccagccccgacacccgccaacacccgctgacgcgccctgacgggcttgtctgctcccggcatccgcttacagacaagctgtgaccgtctccgggagctgcatgtgtcagaggttttcaccgtcatcaccgaaacgcgcgagacgaaagggcctcgtgatacgcctatttttataggttaatgtcatgataataatggtttcttagacgtcaggtggcacttttcggggaaatgtgcgcggaacccctatttgtttatttttctaaatacattcaaatatgtatccgctcatgagacaataaccctgataaatgcttcaataatattgaaaaaggaagagtatgagtattcaacatttccgtgtcgcccttattcccttttttgcggcattttgccttcctgtttttgctcacccagaaacgctggtgaaagtaaaagatgctgaagatcagttgggtgcacgagtgggttacatcgaactggatctcaacagcggtaagatccttgagagttttcgccccgaagaacgttttccaatgatgagcacttttaaagttctgctatgtggcgcggtattatcccgtattgacgccgggcaagagcaactcggtcgccgcatacactattctcagaatgacttggttgagtactcaccagtcacagaaaagcatcttacggatggcatgacagtaagagaattatgcagtgctgccataaccatgagtgataacactgcggccaacttacttctgacaacgatcggaggaccgaaggagctaaccgcttttttgcacaacatgggggatcatgtaactcgccttgatcgttgggaaccggagctgaatgaagccataccaaacgacgagcgtgacaccacgatgcctgtagcaatggcaacaacgttgcgcaaactattaactggcgaactacttactctagcttcccggcaacaattaatagactggatggaggcggataaagttgcaggaccacttctgcgctcggcccttccggctggctggtttattgctgataaatctggagccggtgagcgtgggtctcgcggtatcattgcagcactggggccagatggtaagccctcccgtatcgtagttatctacacgacggggagtcaggcaactatggatgaacgaaatagacagatcgctgagataggtgcctcactgattaagcattggtaactgtcagaccaagtttactcatatatactttagattgatttaaaacttcatttttaatttaaaaggatctaggtgaagatcctttttgataatctcatgaccaaaatcccttaacgtgagttttcgttccactgagcgtcagaccccgtagaaaagatcaaaggatcttcttgagatcctttttttctgcgcgtaatctgctgcttgcaaacaaaaaaaccaccgctaccagcggtggtttgtttgccggatcaagagctaccaactctttttccgaaggtaactggcttcagcagagcgcagataccaaatactgtccttctagtgtagccgtagttaggccaccacttcaagaactctgtagcaccgcctacatacctcgctctgctaatcctgttaccagtggctgctgccagtggcgataagtcgtgtcttaccgggttggactcaagacgatagttaccggataaggcgcagcggtcgggctgaacggggggttcgtgcacacagcccagcttggagcgaacgacctacaccgaactgagatacctacagcgtgagctatgagaaagcgccacgcttcccgaagggagaaaggcggacaggtatccggtaagcggcagggtcggaacaggagagcgcacgagggagcttccagggggaaacgcctggtatctttatagtcctgtcgggtttcgccacctctgacttgagcgtcgatttttgtgatgctcgtcaggggggcggagcctatggaaaaacgccagcaacgcggcctttttacggttcctggccttttgctggccttttgctcacatgttctttcctgcgttatcccctgattctgtggataaccgtattaccgcctttgagtgagctgataccgctcgccgcagccgaacgaccgagcgcagcgagtcagtgagcgaggaagcggaagagcgcccaatacgcaaaccgcctctccccgcgcgttggccgattcattaatg

SEQ ID NO: 39 - protein, 172 aa, Artificial Sequence
  Synthesized
MAAGGPGAGSAAPVSSTSSLPLAALNMRVRRRLSLFLNVRTQVAADWTALAEEMDFEYLEIRQLETQADPTGRLLDAWQGRPGASVGRLLDLLTKLGRDDVLLELGPSIEEDCQKYILKQQQEEAEKPLQVAAVDSSVPRTAELAGITTLDDPLGHMPERFDAFICYCPSDI

SEQ ID NO: 40 - DNA, 8044 bp, Artificial Sequence
  Synthesized
cagcagctggcgtaatagcgaagaggcccgcaccgatcgcccttcccaacagttgcgcagcctgaatggcgaatggaattccagacgattgagcgtcaaaatgtaggtatttccatgagcgtttttcctgttgcaatggctggcggtaatattgttctggatattaccagcaaggccgatagtttgagttcttctactcaggcaagtgatgttattactaatcaaagaagtattgcgacaacggttaatttgcgtgatggacagactcttttactcggtggcctcactgattataaaaacacttctcaggattctggcgtaccgttcctgtctaaaatccctttaatcggcctcctgtttagctcccgctctgattctaacgaggaaagcacgttatacgtgctcgtcaaagcaaccatagtacgcgccctgtagcggcgcattaagcgcggcgggtgtggtggttacgcgcagcgtgaccgctacacttgccagcgccctagcgcccgctcctttcgctttcttcccttcctttctcgccacgttcgccggctttccccgtcaagctctaaatcgggggctccctttagggttccgatttagtgctttacggcacctcgaccccaaaaaacttgattagggtgatggttcacgtagtgggccatcgccctgatagacggtttttcgccctttgacgttggagtccacgttctttaatagtggactcttgttccaaactggaacaacactcaaccctatctcggtctattcttttgatttataagggattttgccgatttcggcctattggttaaaaaatgagctgatttaacaaaaatttaacgcgaattttaacaaaatattaacgtttacaatttaaatatttgcttatacaatcttcctgtttttggggcttttctgattatcaaccggggtacatatgattgacatgctagttttacggcgcgccgggttggccactccctctctgcgcgctcgctcgctcactgaggccgggcgaccaaaggtcgcccgacgcccgggctttgcccgggcggcctcagtgagcgagcgagcgcgcagagagggagtggccaactccatcactaggggttcctacgcgtagatctcatattctggcagggtcagtggctccaactaacatttgtttggtactttacagtttattaaatagatgtttatatggagaagctctcatttctttctcagaagagcctggctaggaaggtggatgaggcaccatattcattttgcaggtgaaattcctgagatgtaaggagctgctgtgacttgctcaaggccttatatcgagtaaacggtagcgctggggcttagacgcaggtgttctgatttatagttcaaaacctctatcaatgagagagcaatctcctggtaatgtgatagatttcccaacttaatgccaacataccataaacctcccattctgctaatgcccagcctaagttggggagaccactccagattccaagatgtacagtttgctttgctgggcctttttcccatgcctgcctttactctgccagagttatattgctggggttttgaagaagatcctattaaataaaagaataagcagtattattaagtagccctgcatttcaggtttccttgagtggcaggccaggcctggccgtgaacgttcactgaaatcatggcctcttggccaagattgatagcttgtgcctgtccctgagtcccagtccatcacgagcagctggtttctaagatgctatttcccgtataaagcatgagaccgtgacttgccagccccacagagccccgcccttgtccatcactggcatctggactccagcctgggttggggcaaagagggaaatgagatcatgtcctaaccctgatcctcttgtcccacagatatccagaaccctgaccctgccgtgtaccagctgagagactctaaatccagtgacaagtctgtctgcctattcaccgattttgattctcaaacaaatgtgtcacaaagtaaggattctgatgtgtatatcacagacaaaactgtgctagacatgaggtctatggacttcaagagcaacagtgctgtggcctggagcaactagtgggcggagttagggcggagccaatcagcgtgcgccgttccgaaagttgccttttatggctgggcggagaatgggcggtgaacgccgatgattatataaggacgcgccgggtgtggcacagctagttccgtcgcagccgggatttgggtcgcggttcttgtttgttccggaaagccaccatggcgctcccagtgacagccttacttttacctctggcgttattattgcacgcggctcgtcctgacatacagatgactcagactacctcttccctatctgcttctttaggcgaccgagtaacaatatcttgccgggccagccaggacatctcaaaatacttaaactggtatcagcagaagccggacggaacagttaagttgctcatttaccacacgtcgagattacactcaggcgttcctagccgattttcgggttccggttccggtacggactacagcctgacaatcagtaaccttgagcaggaggacatcgccacctacttctgtcagcagggcaacacgctcccgtacacattcggtgggggaactaagctggagattaccggaggcggtggcagcggtggcggcggcagcgggggtggcggctcggaggtcaagttacaggagagcggaccgggcttggtcgcacctagccagagcctctcagtcacgtgcactgtgtctggagtcagtctcccagactacggggtatcatggatacgacagccgcctagaaagggcttagagtggctgggggttatctggggaagtgaaaccacatactacaactcagctctcaagagccgcctcaccatcattaaggacaacagtaagtcgcaggttttcttaaagatgaactctctccagactgacgacaccgctatttactactgcgcgaagcactactactacggcgggagttacgcaatggactactggggtcagggcacttctgtgaccgtatccagcactactaccccagccccacgtccccccacgccagctccaacgatagcaagtcagcccttatctcttcgccctgaggcttgcaggcccgcggcgggcggcgccgttcacacgcgaggactagacttcgcctgcgacatctacatctgggcaccactagccgggacttgcggagtgttgttgttgagcttggtaataacgctctactgcatggctgcaggaggtcccggcgcggggtctgcggccccggtctcctccacatcctcccttcccctggctgctctcaacatgcgagtgcggcgccgcctgtctctgttcttgaacgtgcggacacaggtggcggccgactggaccgcgctggcggaggagatggactttgagtacttggagatccggcaactggagacacaagcggaccccactggcaggctgctggacgcctggcagggacgccctggcgcctctgtaggccgactgctcgatctgcttaccaagctgggccgcgacgacgtgctgctggagctgggacccagcattgaggaggattgccaaaagtatatcttgaagcagcagcaggaggaggctgagaagcctttacaggtggccgctgtagacagcagtgtcccacggacagcagagctggcgggcatcaccacacttgatgaccccctggggcatatgcctgagcgtttcgatgccttcatctgctattgccccagcgacatcgtcgagaaagcgagccgcaaaaaagcggcggcggcggcgaaaagcccgtttgcgagcccggcgagcagcgcgcaggaagaagatgcgagcagctgccgcgcgccgagcgaagaagaaggcagctgcgaactgagagtgaagttctctcgctccgcggacgcacccgcttaccagcagggtcagaaccagctatacaacgagttaaacctggggcgccgggaggagtacgacgtgttagacaagcgtagaggtagggacccggagatgggaggcaagcctcggagaaagaacccccaggagggcctgtacaacgaactccagaaggacaagatggctgaggcgtactcggagattggtatgaagggcgagagacgtcgcggaaagggacacgacggcttataccaggggctttccaccgcgaccaaggacacatacgacgcgctgcacatgcaagccttaccacctcgatgaggtaccagcggccgcgatccagacatgataagatacattgatgagtttggacaaaccacaactagaatgcagtgaaaaaaatgctttatttgtgaaatttgtgatgctattgctttatttgtaaccattataagctgcaataaacaagttaacaacaacaattgcattcattttatgtttcaggttcagggggaggtgtgggaggttttttaaagcaagtaaactggtactagtacggatccgcaacaaatctgactttgcatgtgcaaacgccttcaacaacagcattattccagaagacaccttcttccccagcccaggtaagggcagctttggtgccttcgcaggctgtttccttgcttcaggaatggccaggttctgcccagagctctggtcaatgatgtctaaaactcctctgattggtggtctcggccttatccattgccaccaaaaccctctttttactaagaaacagtgagccttgttctggcagtccagagaatgacacgggaaaaaagcagatgaagagaaggtggcaggagagggcacgtggcccagcctcagtctctccaactgagttcctgcctgcctgcctttgctcagactgtttgccccttactgctcttctaggcctcattctaagccccttctccaagttgcctctccttatttctccctgtctgccaaaaaatctttcccagctcactaagtcagtctcacgcagtcactcattaacccaccaatcactgattgtgccggcacatgaatgcaccaggtgttgaagtggaggaattaaaaagtcagatgaggggtgtgcccagaggaagcaccattctagttgggggagcccatctgtcagctgggaaaagtccaaataacttcagattggaatgtgttttaactcagggttgagaaaacagccaccttcaggacaaaagtcagggaagggctctctgaagaaatgctacttgaagataccagccctaccaagggcagggagaggaccaattgatggagttggccactccctctctgcgcgctcgctcgctcactgaggccgcccgggcaaagcccgggcgtcgggcgacctttggtcgcccggcctcagtgagcgagcgagcgcgcagagagggagtggccaacggcgcgcctgcaggttcaaaaatagctaccctctccggcatgaatttatcagctagaacggttgaatatcatattgatggtgatttgactgtctccggcctttctcacccgtttgaatctttacctacacattactcaggcattgcatttaaaatatatgagggttctaaaaatttttatccttgcgttgaaataaaggcttctcccgcaaaagtattacagggtcataatgtttttggtacaaccgatttagctttatgctctgaggctttattgcttaattttgctaattctttgccttgcctgtatgatttattggatgttggaattcctgatgcggtattttctccttacgcatctgtgcggtatttcacaccgcatatggtgcactctcagtacaatctgctctgatgccgcatagttaagccagccccgacacccgccaacacccgctgacgcgccctgacgggcttgtctgctcccggcatccgcttacagacaagctgtgaccgtctccgggagctgcatgtgtcagaggttttcaccgtcatcaccgaaacgcgcgagacgaaagggcctcgtgatacgcctatttttataggttaatgtcatgataataatggtttcttagacgtcaggtggcacttttcggggaaatgtgcgcggaacccctatttgtttatttttctaaatacattcaaatatgtatccgctcatgagacaataaccctgataaatgcttcaataatattgaaaaaggaagagtatgagtattcaacatttccgtgtcgcccttattcccttttttgcggcattttgccttcctgtttttgctcacccagaaacgctggtgaaagtaaaagatgctgaagatcagttgggtgcacgagtgggttacatcgaactggatctcaacagcggtaagatccttgagagttttcgccccgaagaacgttttccaatgatgagcacttttaaagttctgctatgtggcgcggtattatcccgtattgacgccgggcaagagcaactcggtcgccgcatacactattctcagaatgacttggttgagtactcaccagtcacagaaaagcatcttacggatggcatgacagtaagagaattatgcagtgctgccataaccatgagtgataacactgcggccaacttacttctgacaacgatcggaggaccgaaggagctaaccgcttttttgcacaacatgggggatcatgtaactcgccttgatcgttgggaaccggagctgaatgaagccataccaaacgacgagcgtgacaccacgatgcctgtagcaatggcaacaacgttgcgcaaactattaactggcgaactacttactctagcttcccggcaacaattaatagactggatggaggcggataaagttgcaggaccacttctgcgctcggcccttccggctggctggtttattgctgataaatctggagccggtgagcgtgggtctcgcggtatcattgcagcactggggccagatggtaagccctcccgtatcgtagttatctacacgacggggagtcaggcaactatggatgaacgaaatagacagatcgctgagataggtgcctcactgattaagcattggtaactgtcagaccaagtttactcatatatactttagattgatttaaaacttcatttttaatttaaaaggatctaggtgaagatcctttttgataatctcatgaccaaaatcccttaacgtgagttttcgttccactgagcgtcagaccccgtagaaaagatcaaaggatcttcttgagatcctttttttctgcgcgtaatctgctgcttgcaaacaaaaaaaccaccgctaccagcggtggtttgtttgccggatcaagagctaccaactctttttccgaaggtaactggcttcagcagagcgcagataccaaatactgtccttctagtgtagccgtagttaggccaccacttcaagaactctgtagcaccgcctacatacctcgctctgctaatcctgttaccagtggctgctgccagtggcgataagtcgtgtcttaccgggttggactcaagacgatagttaccggataaggcgcagcggtcgggctgaacggggggttcgtgcacacagcccagcttggagcgaacgacctacaccgaactgagatacctacagcgtgagctatgagaaagcgccacgcttcccgaagggagaaaggcggacaggtatccggtaagcggcagggtcggaacaggagagcgcacgagggagcttccagggggaaacgcctggtatctttatagtcctgtcgggtttcgccacctctgacttgagcgtcgatttttgtgatgctcgtcaggggggcggagcctatggaaaaacgccagcaacgcggcctttttacggttcctggccttttgctggccttttgctcacatgttctttcctgcgttatcccctgattctgtggataaccgtattaccgcctttgagtgagctgataccgctcgccgcagccgaacgaccgagcgcagcgagtcagtgagcgaggaagcggaagagcgcccaatacgcaaaccgcctctccccgcgcgttggccgattcattaatg

SEQ ID NO: 41 - protein, 216 aa, Artificial Sequence
  Synthesized
GVQVETISPGDGRTFPKRGQTCVVHYTGMLEDGKKVDSSRDRNKPFKFMLGKQEVIRGWEEGVAQMSVGQRAKLTISPDYAYGATGHPGIIPPHATLVFDVELLKLEVEGVQVETISPGDGRTFPKRGQTCVVHYTGMLEDGKKVDSSRDRNKPFKFMLGKQEVIRGWEEGVAQMSVGQRAKLTISPDYAYGATGHPGIIPPHATLVFDVELLKLE

SEQ ID NO: 42 - DNA, 7760 bp, Artificial Sequence
  Synthesized
cagcagctggcgtaatagcgaagaggcccgcaccgatcgcccttcccaacagttgcgcagcctgaatggcgaatggaattccagacgattgagcgtcaaaatgtaggtatttccatgagcgtttttcctgttgcaatggctggcggtaatattgttctggatattaccagcaaggccgatagtttgagttcttctactcaggcaagtgatgttattactaatcaaagaagtattgcgacaacggttaatttgcgtgatggacagactcttttactcggtggcctcactgattataaaaacacttctcaggattctggcgtaccgttcctgtctaaaatccctttaatcggcctcctgtttagctcccgctctgattctaacgaggaaagcacgttatacgtgctcgtcaaagcaaccatagtacgcgccctgtagcggcgcattaagcgcggcgggtgtggtggttacgcgcagcgtgaccgctacacttgccagcgccctagcgcccgctcctttcgctttcttcccttcctttctcgccacgttcgccggctttccccgtcaagctctaaatcgggggctccctttagggttccgatttagtgctttacggcacctcgaccccaaaaaacttgattagggtgatggttcacgtagtgggccatcgccctgatagacggtttttcgccctttgacgttggagtccacgttctttaatagtggactcttgttccaaactggaacaacactcaaccctatctcggtctattcttttgatttataagggattttgccgatttcggcctattggttaaaaaatgagctgatttaacaaaaatttaacgcgaattttaacaaaatattaacgcttacaatttaaatatttgcttatacaatcttcctgtttttggggcttttctgattatcaaccggggtacatatgattgacatgctagttttacggcgcgccgggttggccactccctctctgcgcgctcgctcgctcactgaggccgggcgaccaaaggtcgcccgacgcccgggctttgcccgggcggcctcagtgagcgagcgagcgcgcagagagggagtggccaactccatcactaggggttcctacgcgtagatctcatcacgagcagctggtttctaagatgctatttcccgtataaagcatgagaccgtgacttgccagccccacagagccccgcccttgtccatcactggcatctggactccagcctgggttggggcaaagagggaaatgagatcatgtcctaaccctgatcctcttgtcccacagatatccagaaccctgaccctgccgtgtaccagctgagagactctaaatccagtgacaagtctgtctgcctattcaccgattttgattctcaaacaaatgtgtcacaaagtaaggattctgatgtgtatatcacagacaaaactgtgctagacatgaggtctatggacttcaagagcaacagtgctgtggcctggagcaactagtgggcggagttagggcggagccaatcagcgtgcgccgttccgaaagttgccttttatggctgggcggagaatgggcggtgaacgccgatgattatataaggacgcgccgggtgtggcacagctagttccgtcgcagccgggatttgggtcgcggttcttgtttgttccctcgagccaccatggctgcaggaggtcccggcgcggggtctgcggccccggtctcctccacatcctcccttcccctggctgctctcaacatgcgagtgcggcgccgcctgtctctgttcttgaacgtgcggacacaggtggcggccgactggaccgcgctggcggaggagatggactttgagtacttggagatccggcaactggagacacaagcggaccccactggcaggctgctggacgcctggcagggacgccctggcgcctctgtaggccgactgctcgatctgcttaccaagctgggccgcgacgacgtgctgctggagctgggacccagcattgaggaggattgccaaaagtatatcttgaagcagcagcaggaggaggctgagaagcctttacaggtggccgctgtagacagcagtgtcccacggacagcagagctggcgggcatcaccacacttgatgaccccctggggcatatgcctgagcgtttcgatgccttcatctgctattgccccagcgacatcgtcgagaaagcgagccgcaaaaaagcggcggcggcggcgaaaagcccgtttgcgagcccggcgagcagcgcgcaggaagaagatgcgagcagctgccgcgcgccgagcgaagaagaaggcagctgcgaactggtcgagggcgtccaagtcgaaaccattagtcccggcgatggcagaacatttcctaaaaggggacaaacatgtgtcgtccattatacaggcatgttggaggacggcaaaaaggtggacagtagtagagatcgcaataaacctttcaaattcatgttgggaaaacaagaagtcattaggggatgggaggagggcgtggctcaaatgtccgtcggccaacgcgctaagctcaccatcagccccgactacgcatacggcgctaccggacatcccggaattattccccctcacgctaccttggtgtttgacgtcgaactgttgaagctcgaagtcgagggagtgcaggtggagactatctccccaggagacgggcgcaccttccccaagcgcggccagacctgcgtggtgcactacaccgggatgcttgaagatggaaagaaagttgattcctcccgggacagaaacaagccctttaagtttatgctaggcaagcaggaggtgatccgaggctgggaagaaggggttgcccagatgagtgtgggtcagagagccaaactgactatatctccagattatgcctatggtgccactgggcacccaggcatcatcccaccacatgccactctcgtcttcgatgtggagcttctaaaactggaaccgcgggaaggccgagggagcctgctgacatgtggcgatgtggaggaaaacccaggaccaccatggatggcgctcccagtgacagccttacttttacctctggcgttattattgcacgcggctcgtcctgacatacagatgactcagactacctcttccctatctgcttctttaggcgaccgagtaacaatatcttgccgggccagccaggacatctcaaaatacttaaactggtatcagcagaagccggacggaacagttaagttgctcatttaccacacgtcgagattacactcaggcgttcctagccgattttcgggttccggttccggtacggactacagcctgacaatcagtaaccttgagcaggaggacatcgccacctacttctgtcagcagggcaacacgctcccgtacacattcggtgggggaactaagctggagattaccggaggcggtggcagcggtggcggcggcagcgggggtggcggctcggaggtcaagttacaggagagcggaccgggcttggtcgcacctagccagagcctctcagtcacgtgcactgtgtctggagtcagtctcccagactacggggtatcatggatacgacagccgcctagaaagggcttagagtggctgggggttatctggggaagtgaaaccacatactacaactcagctctcaagagccgcctcaccatcattaaggacaacagtaagtcgcaggttttcttaaagatgaactctctccagactgacgacaccgctatttactactgcgcgaagcactactactacggcgggagttacgcaatggactactggggtcagggcacttctgtgaccgtatccagcactactaccccagccccacgtccccccacgccagctccaacgatagcaagtcagcccttatctcttcgccctgaggcttgcaggcccgcggcgggcggcgccgttcacacgcgaggactagacttcgcctgcgacatctacatctgggcaccactagccgggacttgcggagtgttgttgttgagcttggtaataacgctctactgcagagtgaagttctctcgctccgcggacgcacccgcttaccagcagggtcagaaccagctatacaacgagttaaacctggggcgccgggaggagtacgacgtgttagacaagcgtagaggtagggacccggagatgggaggcaagcctcggagaaagaacccccaggagggcctgtacaacgaactccagaaggacaagatggctgaggcgtactcggagattggtatgaagggcgagagacgtcgcggaaagggacacgacggcttataccaggggctttccaccgcgaccaaggacacatacgacgcgctgcacatgcaagccttaccacctcgatgaggtaccagcgcggccgcgatccagacatgataagatacattgatgagtttggacaaaccacaactagaatgcagtgaaaaaaatgctttatttgtgaaatttgtgatgctattgctttatttgtaaccattataagctgcaataaacaagttaacaacaacaattgcattcattttatgtttcaggttcagggggaggtgtgggaggttttttaaagcaagtaaactggtactagtacggatccgcaacaaatctgactttgcatgtgcaaacgccttcaacaacagcattattccagaagacaccttcttccccagcccaggtaagggcagctttggtgccttcgcaggctgtttccttgcttcaggaatggccaggttctgcccagagctctggtcaatgatgtctaaaactcctctgattggtggtctcggccttatccattgccaccaaaaccctctttttactaagaaacagtgagccttgttctggcagtccagagaatgacacgggaaaaaagcagatgaagagaaggtggcaggagagggcacgtggcccagcctcagtctctccaactgagttcctgcctgcctgcctttgctcagactgtttgcccaattgatggagttggccactccctctctgcgcgctcgctcgctcactgaggccgcccgggcaaagcccgggcgtcgggcgacctttggtcgcccggcctcagtgagcgagcgagcgcgcagagagggagtggccaacggcgcgcctgcaggttcaaaaatagctaccctctccggcatgaatttatcagctagaacggttgaatatcatattgatggtgatttgactgtctccggcctttctcacccgtttgaatctttacctacacattactcaggcattgcatttaaaatatatgagggttctaaaaatttttatccttgcgttgaaataaaggcttctcccgcaaaagtattacagggtcataatgtttttggtacaaccgatttagctttatgctctgaggctttattgcttaattttgctaattctttgccttgcctgtatgatttattggatgttggaattcctgatgcggtattttctccttacgcatctgtgcggtatttcacaccgcatatggtgcactctcagtacaatctgctctgatgccgcatagttaagccagccccgacacccgccaacacccgctgacgcgccctgacgggcttgtctgctcccggcatccgcttacagacaagctgtgaccgtctccgggagctgcatgtgtcagaggttttcaccgtcatcaccgaaacgcgcgagacgaaagggcctcgtgatacgcctatttttataggttaatgtcatgataataatggtttcttagacgtcaggtggcacttttcggggaaatgtgcgcggaacccctatttgtttatttttctaaatacattcaaatatgtatccgctcatgagacaataaccctgataaatgcttcaataatattgaaaaaggaagagtatgagtattcaacatttccgtgtcgcccttattcccttttttgcggcattttgccttcctgtttttgctcacccagaaacgctggtgaaagtaaaagatgctgaagatcagttgggtgcacgagtgggttacatcgaactggatctcaacagcggtaagatccttgagagttttcgccccgaagaacgttttccaatgatgagcacttttaaagttctgctatgtggcgcggtattatcccgtattgacgccgggcaagagcaactcggtcgccgcatacactattctcagaatgacttggttgagtactcaccagtcacagaaaagcatcttacggatggcatgacagtaagagaattatgcagtgctgccataaccatgagtgataacactgcggccaacttacttctgacaacgatcggaggaccgaaggagctaaccgcttttttgcacaacatgggggatcatgtaactcgccttgatcgttgggaaccggagctgaatgaagccataccaaacgacgagcgtgacaccacgatgcctgtagcaatggcaacaacgttgcgcaaactattaactggcgaactacttactctagcttcccggcaacaattaatagactggatggaggcggataaagttgcaggaccacttctgcgctcggcccttccggctggctggtttattgctgataaatctggagccggtgagcgtgggtctcgcggtatcattgcagcactggggccagatggtaagccctcccgtatcgtagttatctacacgacggggagtcaggcaactatggatgaacgaaatagacagatcgctgagataggtgcctcactgattaagcattggtaactgtcagaccaagtttactcatatatactttagattgatttaaaacttcatttttaatttaaaaggatctaggtgaagatcctttttgataatctcatgaccaaaatcccttaacgtgagttttcgttccactgagcgtcagaccccgtagaaaagatcaaaggatcttcttgagatcctttttttctgcgcgtaatctgctgcttgcaaacaaaaaaaccaccgctaccagcggtggtttgtttgccggatcaagagctaccaactctttttccgaaggtaactggcttcagcagagcgcagataccaaatactgtccttctagtgtagccgtagttaggccaccacttcaagaactctgtagcaccgcctacatacctcgctctgctaatcctgttaccagtggctgctgccagtggcgataagtcgtgtcttaccgggttggactcaagacgatagttaccggataaggcgcagcggtcgggctgaacggggggttcgtgcacacagcccagcttggagcgaacgacctacaccgaactgagatacctacagcgtgagctatgagaaagcgccacgcttcccgaagggagaaaggcggacaggtatccggtaagcggcagggtcggaacaggagagcgcacgagggagcttccagggggaaacgcctggtatctttatagtcctgtcgggtttcgccacctctgacttgagcgtcgatttttgtgatgctcgtcaggggggcggagcctatggaaaaacgccagcaacgcggcctttttacggttcctggccttttgctggccttttgctcacatgttctttcctgcgttatcccctgattctgtggataaccgtattaccgcctttgagtgagctgataccgctcgccgcagccgaacgaccgagcgcagcgagtcagtgagcgaggaagcggaagagcgcccaatacgcaaaccgcctctccccgcgcgttggccgattcattaatg